European Patent Specification EP 3 368 555 B1, published January 15, 2025. Title: DUAL FUNCTION PROTEINS AND PHARMACEUTICAL COMPOSITION COMPRISING SAME. Applicant: YUHAN CORPORATION. The sequence listing filed with the application follows.

SEQUENCE LISTING (80 sequences)

SEQ ID NO: 1 - protein, 181 aa, human FGF21
HPIPDSSPLLQFGGQVRQRYLYTDDAQQTEAHLEIREDGTVGGAADQSPESLLQLKALKPGVIQILGVKTSRFLCQRPDGALYGSLHFDPEACSFRELLLEDGYNVYQSEAHGLPLHLPGNKSPHRDPAPRGPARFLPLPGLPPALPEPPGILAPQPPDVGSSDPLSMVGPSQGRSPSYAS

SEQ ID NO: 2 - protein, 30 aa, Artificial Sequence
  linker
AKATTAPATTRNTGRGGEEKKKEKEKEEQE

SEQ ID NO: 3 - protein, 17 aa, Artificial Sequence
  linker
AKATTAPATTRNTGRGG

SEQ ID NO: 4 - protein, 15 aa, Artificial Sequence
  linker
GGGGSGGGGSGGGGS

SEQ ID NO: 5 - protein, 16 aa, Artificial Sequence
  linker
GGGGSGGGGSGGGGSA

SEQ ID NO: 6 - protein, 181 aa, Artificial Sequence
  FGF21 variant
HPIPDSSPLLQFGGQVRQRYLYTDDAQQTEAHLEIREDGTVGGAADQSPESLLQLKALKPGVIQILGVKTSRFLCQRPDGALYGSLHFDPEACSFREEIRPDGYNVYQSEAHGLPLHLPGNKSPHRDPAPRGPARFLPLPGLPPALPEPPGILAPQPPDVGSSDPLSMVGPSQGRSPSYAS

SEQ ID NO: 7 - protein, 182 aa, Artificial Sequence
  FGF21 variant
HPIPDSSPLLQFGGQVRQRYLYTDDAQQTEAHLEIREDGTVGGAADQSPESLLQLKALKPGVIQILGVKTSRFLCQRPDGALYGSLHFDPEACSFRELLLEDGYNVYQSEAHGLPLHLPGNKSPHRDPAPRGPARFLPLPGLPPALPEPPGILAPQPPDVGSSDPLSMVTGLEAVRSPSYAS

SEQ ID NO: 8 - protein, 182 aa, Artificial Sequence
  FGF21 variant
HPIPDSSPLLQFGGQVRQRYLYTDDAQQTEAHLEIREDGTVGGAADQSPESLLQLKALKPGVIQILGVKTSRFLCQRPDGALYGSLHFDPEACSFRELLLEDGYNVYQSEAHGLPLHLPGNKSPHRDPAPRGPARFLPLPGLPPALPEPPGILAPQPPDVGSSDPLSMVTGLEANRSPSYAS

SEQ ID NO: 9 - protein, 181 aa, Artificial Sequence
  FGF21 variant
HPIPDSSPLLQFGGQVRQRYLYTDDAQQTEAHLEIREDGTVGGAADQSPESLLQLKALKPGVIQILGVKTSRFLCQRPDGALYGSLHFDPEACSFRELLLEDGYNVYQSEAHGLPLHLPGNKSPHRDPAPRGPARFLPLPGLPPALPEPPGILAPQPPDVGSSDPLSMVNPSQGRSPSYAS

SEQ ID NO: 10 - protein, 181 aa, Artificial Sequence
  FGF21 variant
HPIPDSSPLLQFGGQVRQRYLYTDDAQQTEAHLEIREDGTVGGAADQSPESLLQLKALKPGVIQILGVKTSRFLCQRPDGALYGSLHFDPEACSFRELLLEDGYNVYQSEAHGLPLHLPGNKSPHRDPAPRGPARFLPLPGLPPALPEPPGILAPQPPDVGSSDPLSMVGPSQNRSPSYAS

SEQ ID NO: 11 - protein, 182 aa, Artificial Sequence
  FGF21 variant
HPIPDSSPLLQFGGQVRQRYLYTDDAQQTEAHLEIREDGTVGGAADQSPESLLQLKALKPGVIQILGVKTSRFLCQRPDGALYGSLHFDPEACSFREEIRPDGYNVYQSEAHGLPLHLPGNKSPHRDPAPRGPARFLPLPGLPPALPEPPGILAPQPPDVGSSDPLSMVTGLEAVRSPSYAS

SEQ ID NO: 12 - protein, 182 aa, Artificial Sequence
  FGF21 variant
HPIPDSSPLLQFGGQVRQRYLYTDDAQQTEAHLEIREDGTVGGAADQSPESLLQLKALKPGVIQILGVKTSRFLCQRPDGALYGSLHFDPEACSFREEIRPDGYNVYQSEAHGLPLHLPGNKSPHRDPAPRGPARFLPLPGLPPALPEPPGILAPQPPDVGSSDPLSMVTGLEANRSPSYAS

SEQ ID NO: 13 - protein, 181 aa, Artificial Sequence
  FGF21 variant
HPIPDSSPLLQFGGQVRQRYLYTDDAQQTEAHLEIREDGTVGGAADQSPESLLQLKALKPGVIQILGVKTSRFLCQRPDGALYGSLHFDPEACSFREEIRPDGYNVYQSEAHGLPLHLPGNKSPHRDPAPRGPARFLPLPGLPPALPEPPGILAPQPPDVGSSDPLSMVNPSQGRSPSYAS

SEQ ID NO: 14 - protein, 181 aa, Artificial Sequence
  FGF21 variant
HPIPDSSPLLQFGGQVRQRYLYTDDAQQTEAHLEIREDGTVGGAADQSPESLLQLKALKPGVIQILGVKTSRFLCQRPDGALYGSLHFDPEACSFREEIRPDGYNVYQSEAHGLPLHLPGNKSPHRDPAPRGPARFLPLPGLPPALPEPPGILAPQPPDVGSSDPLSMVGPSQNRSPSYAS

SEQ ID NO: 15 - protein, 181 aa, Artificial Sequence
  FGF21 variant
HPIPDSSPLLQFGGQVRQRYLYTDDAQQTEAHLEIREDGTVGGAADQSPESLLQLKALKPGVIQILGVKTSRFLCQRPDGALYGSLHFDPEACSFREEIRPDGYNVYQSEAHGLPLHLPGNKSPHRDPAPRGPARFLPLPGLPPALPEPPGILAPQPPDVGSSDPLSMVGPSQGRSPSYES

SEQ ID NO: 16 - protein, 182 aa, Artificial Sequence
  FGF21 variant
HPIPDSSPLLQFGGQVRQRYLYTDDAQQTEAHLEIREDGTVGGAADQSPESLLQLKALKPGVIQILGVKTSRFLCQRPDGALYGSLHFDPEACSFRELLLEDGYNVYQSEAHGLPLHLPGNKSPHRDPAPRGPARFLPLPGLPPALPEPPGILAPQPPDVGSSDPLSMVTGLEAVRSPSYES

SEQ ID NO: 17 - protein, 182 aa, Artificial Sequence
  FGF21 variant
HPIPDSSPLLQFGGQVRQRYLYTDDAQQTEAHLEIREDGTVGGAADQSPESLLQLKALKPGVIQILGVKTSRFLCQRPDGALYGSLHFDPEACSFRELLLEDGYNVYQSEAHGLPLHLPGNKSPHRDPAPRGPARFLPLPGLPPALPEPPGILAPQPPDVGSSDPLSMVTGLEANRSPSYES

SEQ ID NO: 18 - protein, 181 aa, Artificial Sequence
  FGF21 variant
HPIPDSSPLLQFGGQVRQRYLYTDDAQQTEAHLEIREDGTVGGAADQSPESLLQLKALKPGVIQILGVKTSRFLCQRPDGALYGSLHFDPEACSFRELLLEDGYNVYQSEAHGLPLHLPGNKSPHRDPAPRGPARFLPLPGLPPALPEPPGILAPQPPDVGSSDPLSMVNPSQGRSPSYES

SEQ ID NO: 19 - protein, 181 aa, Artificial Sequence
  FGF21 variant
HPIPDSSPLLQFGGQVRQRYLYTDDAQQTEAHLEIREDGTVGGAADQSPESLLQLKALKPGVIQILGVKTSRFLCQRPDGALYGSLHFDPEACSFRELLLEDGYNVYQSEAHGLPLHLPGNKSPHRDPAPRGPARFLPLPGLPPALPEPPGILAPQPPDVGSSDPLSMVGPSQNRSPSYES

SEQ ID NO: 20 - protein, 182 aa, Artificial Sequence
  FGF21 variant
HPIPDSSPLLQFGGQVRQRYLYTDDAQQTEAHLEIREDGTVGGAADQSPESLLQLKALKPGVIQILGVKTSRFLCQRPDGALYGSLHFDPEACSFREEIRPDGYNVYQSEAHGLPLHLPGNKSPHRDPAPRGPARFLPLPGLPPALPEPPGILAPQPPDVGSSDPLSMVTGLEAVRSPSYES

SEQ ID NO: 21 - protein, 182 aa, Artificial Sequence
  FGF21 variant
HPIPDSSPLLQFGGQVRQRYLYTDDAQQTEAHLEIREDGTVGGAADQSPESLLQLKALKPGVIQILGVKTSRFLCQRPDGALYGSLHFDPEACSFREEIRPDGYNVYQSEAHGLPLHLPGNKSPHRDPAPRGPARFLPLPGLPPALPEPPGILAPQPPDVGSSDPLSMVTGLEANRSPSYES

SEQ ID NO: 22 - protein, 181 aa, Artificial Sequence
  FGF21 variant
HPIPDSSPLLQFGGQVRQRYLYTDDAQQTEAHLEIREDGTVGGAADQSPESLLQLKALKPGVIQILGVKTSRFLCQRPDGALYGSLHFDPEACSFREEIRPDGYNVYQSEAHGLPLHLPGNKSPHRDPAPRGPARFLPLPGLPPALPEPPGILAPQPPDVGSSDPLSMVNPSQGRSPSYES

SEQ ID NO: 23 - protein, 181 aa, Artificial Sequence
  FGF21 variant
HPIPDSSPLLQFGGQVRQRYLYTDDAQQTEAHLEIREDGTVGGAADQSPESLLQLKALKPGVIQILGVKTSRFLCQRPDGALYGSLHFDPEACSFREEIRPDGYNVYQSEAHGLPLHLPGNKSPHRDPAPRGPARFLPLPGLPPALPEPPGILAPQPPDVGSSDPLSMVGPSQNRSPSYES

SEQ ID NO: 24 - protein, 229 aa, Artificial Sequence
  Human IgG4 Fc
ESKYGPPCPSCPAPEFLGGPSVFLFPPKPKDTLMISRTPEVTCVVVDVSQEDPEVQFNWYVDGVEVHNAKTKPREEQFNSTYRVVSVLTVLHQDWLNGKEYKCKVSNKGLPSSIEKTISKAKGQPREPQVYTLPPSQEEMTKNQVSLTCLVKGFYPSDIAVEWESNGQPENNYKTTPPVLDSDGSFFLYSRLTVDKSRWQEGNVFSCSVMHEALHNHYTQKSLSLSLGK

SEQ ID NO: 25 - protein, 228 aa, Artificial Sequence
  Human IgG4 Fc variant
ESKYGPPCPPCPAPEAAGGPSVFLFPPKPKDTLMISRTPEVTCVVVDVSQEDPEVQFNWYVDGVEVHNAKTKPREEQFNSTYRVVSVLTVLHQDWLNGKEYKCKVSNKGLPSSIEKTISKAKGQPREPQVYTLPPSQEEMTKNQVSLTCLVKGFYPSDIAVEWESNGQPENNYKTTPPVLDSDGSFFLYSRLTVDKSRWQEGNVFSCSVMHEALHNHYTQKSLSLSLG

SEQ ID NO: 26 - protein, 223 aa, Artificial Sequence
  Hybrid Fc variant
ETKTPECPSHTQPLGVFLFPPKPKDTLMISRTPEVTCVVVDVSQEDPEVQFNWYVDGVEVHNAKTKPREEQFNSTYRVVSVLTVLHQDWLNGKEYKCKVSNKGLPSSIEKTISKAKGQPREPQVYTLPPSQEEMTKNQVSLTCLVKGFYPSDIAVEWESNGQPENNYKTTPPVLDSDGSFFLYSRLTVDKSRWQEGNVFSCSVMHEALHNHYTQKSLSLSLGK

SEQ ID NO: 27 - protein, 435 aa, Artificial Sequence
  modified FGF21 variant connected to hybrid Fc
ETKTPECPSHTQPLGVFLFPPKPKDTLMISRTPEVTCVVVDVSQEDPEVQFNWYVDGVEVHNAKTKPREEQFNSTYRVVSVLTVLHQDWLNGKEYKCKVSNKGLPSSIEKTISKAKGQPREPQVYTLPPSQEEMTKNQVSLTCLVKGFYPSDIAVEWESNGQPENNYKTTPPVLDSDGSFFLYSRLTVDKSRWQEGNVFSCSVMHEALHNHYTQKSLSLSLGKAKATTAPATTRNTGRGGEEKKKEKEKEEQEHPIPDSSPLLQFGGQVRQRYLYTDDAQQTEAHLEIREDGTVGGAADQSPESLLQLKALKPGVIQILGVKTSRFLCQRPDGALYGSLHFDPEACSFREEIRPDGYNVYQSEAHGLPLHLPGNKSPHRDPAPRGPARFLPLPGLPPALPEPPGILAPQPPDVGSSDPLSMVTGLEAVRSPSYAS

SEQ ID NO: 28 - protein, 422 aa, Artificial Sequence
  modified FGF21 variant connected to hybrid Fc
ETKTPECPSHTQPLGVFLFPPKPKDTLMISRTPEVTCVVVDVSQEDPEVQFNWYVDGVEVHNAKTKPREEQFNSTYRVVSVLTVLHQDWLNGKEYKCKVSNKGLPSSIEKTISKAKGQPREPQVYTLPPSQEEMTKNQVSLTCLVKGFYPSDIAVEWESNGQPENNYKTTPPVLDSDGSFFLYSRLTVDKSRWQEGNVFSCSVMHEALHNHYTQKSLSLSLGKAKATTAPATTRNTGRGGHPIPDSSPLLQFGGQVRQRYLYTDDAQQTEAHLEIREDGTVGGAADQSPESLLQLKALKPGVIQILGVKTSRFLCQRPDGALYGSLHFDPEACSFRELLLEDGYNVYQSEAHGLPLHLPGNKSPHRDPAPRGPARFLPLPGLPPALPEPPGILAPQPPDVGSSDPLSMVTGLEAVRSPSYAS

SEQ ID NO: 29 - protein, 420 aa, Artificial Sequence
  modified FGF21 variant connected to hybrid Fc
ETKTPECPSHTQPLGVFLFPPKPKDTLMISRTPEVTCVVVDVSQEDPEVQFNWYVDGVEVHNAKTKPREEQFNSTYRVVSVLTVLHQDWLNGKEYKCKVSNKGLPSSIEKTISKAKGQPREPQVYTLPPSQEEMTKNQVSLTCLVKGFYPSDIAVEWESNGQPENNYKTTPPVLDSDGSFFLYSRLTVDKSRWQEGNVFSCSVMHEALHNHYTQKSLSLSLGKGGGGSGGGGSGGGGSHPIPDSSPLLQFGGQVRQRYLYTDDAQQTEAHLEIREDGTVGGAADQSPESLLQLKALKPGVIQILGVKTSRFLCQRPDGALYGSLHFDPEACSFRELLLEDGYNVYQSEAHGLPLHLPGNKSPHRDPAPRGPARFLPLPGLPPALPEPPGILAPQPPDVGSSDPLSMVTGLEAVRSPSYAS

SEQ ID NO: 30 - protein, 420 aa, Artificial Sequence
  modified FGF21 variant connected to hybrid Fc
ETKTPECPSHTQPLGVFLFPPKPKDTLMISRTPEVTCVVVDVSQEDPEVQFNWYVDGVEVHNAKTKPREEQFNSTYRVVSVLTVLHQDWLNGKEYKCKVSNKGLPSSIEKTISKAKGQPREPQVYTLPPSQEEMTKNQVSLTCLVKGFYPSDIAVEWESNGQPENNYKTTPPVLDSDGSFFLYSRLTVDKSRWQEGNVFSCSVMHEALHNHYTQKSLSLSLGKGGGGSGGGGSGGGGSHPIPDSSPLLQFGGQVRQRYLYTDDAQQTEAHLEIREDGTVGGAADQSPESLLQLKALKPGVIQILGVKTSRFLCQRPDGALYGSLHFDPEACSFRELLLEDGYNVYQSEAHGLPLHLPGNKSPHRDPAPRGPARFLPLPGLPPALPEPPGILAPQPPDVGSSDPLSMVTGLEANRSPSYAS

SEQ ID NO: 31 - protein, 419 aa, Artificial Sequence
  modified FGF21 variant connected to hybrid Fc
ETKTPECPSHTQPLGVFLFPPKPKDTLMISRTPEVTCVVVDVSQEDPEVQFNWYVDGVEVHNAKTKPREEQFNSTYRVVSVLTVLHQDWLNGKEYKCKVSNKGLPSSIEKTISKAKGQPREPQVYTLPPSQEEMTKNQVSLTCLVKGFYPSDIAVEWESNGQPENNYKTTPPVLDSDGSFFLYSRLTVDKSRWQEGNVFSCSVMHEALHNHYTQKSLSLSLGKGGGGSGGGGSGGGGSHPIPDSSPLLQFGGQVRQRYLYTDDAQQTEAHLEIREDGTVGGAADQSPESLLQLKALKPGVIQILGVKTSRFLCQRPDGALYGSLHFDPEACSFRELLLEDGYNVYQSEAHGLPLHLPGNKSPHRDPAPRGPARFLPLPGLPPALPEPPGILAPQPPDVGSSDPLSMVNPSQGRSPSYAS

SEQ ID NO: 32 - protein, 419 aa, Artificial Sequence; identical to SEQ ID NO: 31
  modified FGF21 variant connected to hybrid Fc

SEQ ID NO: 33 - protein, 419 aa, Artificial Sequence
  modified FGF21 variant connected to hybrid Fc
ETKTPECPSHTQPLGVFLFPPKPKDTLMISRTPEVTCVVVDVSQEDPEVQFNWYVDGVEVHNAKTKPREEQFNSTYRVVSVLTVLHQDWLNGKEYKCKVSNKGLPSSIEKTISKAKGQPREPQVYTLPPSQEEMTKNQVSLTCLVKGFYPSDIAVEWESNGQPENNYKTTPPVLDSDGSFFLYSRLTVDKSRWQEGNVFSCSVMHEALHNHYTQKSLSLSLGKGGGGSGGGGSGGGGSHPIPDSSPLLQFGGQVRQRYLYTDDAQQTEAHLEIREDGTVGGAADQSPESLLQLKALKPGVIQILGVKTSRFLCQRPDGALYGSLHFDPEACSFRELLLEDGYNVYQSEAHGLPLHLPGNKSPHRDPAPRGPARFLPLPGLPPALPEPPGILAPQPPDVGSSDPLSMVGPSQNRSPSYAS

SEQ ID NO: 34 - protein, 419 aa, Artificial Sequence
  modified FGF21 variant connected to hybrid Fc
ETKTPECPSHTQPLGVFLFPPKPKDTLMISRTPEVTCVVVDVSQEDPEVQFNWYVDGVEVHNAKTKPREEQFNSTYRVVSVLTVLHQDWLNGKEYKCKVSNKGLPSSIEKTISKAKGQPREPQVYTLPPSQEEMTKNQVSLTCLVKGFYPSDIAVEWESNGQPENNYKTTPPVLDSDGSFFLYSRLTVDKSRWQEGNVFSCSVMHEALHNHYTQKSLSLSLGKGGGGSGGGGSGGGGSHPIPDSSPLLQFGGQVRQRYLYTDDAQQTEAHLEIREDGTVGGAADQSPESLLQLKALKPGVIQILGVKTSRFLCQRPDGALYGSLHFDPEACSFRELLLEDGYNVYQSEAHGLPLHLPGNKSPHRDPAPRGPARFLPLPGLPPALPEPPGILAPQPPDVGSSDPLSMVGPSQGRSPSYAS

SEQ ID NO: 35 - protein, 420 aa, Artificial Sequence
  modified FGF21 variant connected to hybrid Fc
ETKTPECPSHTQPLGVFLFPPKPKDTLMISRTPEVTCVVVDVSQEDPEVQFNWYVDGVEVHNAKTKPREEQFNSTYRVVSVLTVLHQDWLNGKEYKCKVSNKGLPSSIEKTISKAKGQPREPQVYTLPPSQEEMTKNQVSLTCLVKGFYPSDIAVEWESNGQPENNYKTTPPVLDSDGSFFLYSRLTVDKSRWQEGNVFSCSVMHEALHNHYTQKSLSLSLGKGGGGSGGGGSGGGGSHPIPDSSPLLQFGGQVRQRYLYTDDAQQTEAHLEIREDGTVGGAADQSPESLLQLKALKPGVIQILGVKTSRFLCQRPDGALYGSLHFDPEACSFREEIRPDGYNVYQSEAHGLPLHLPGNKSPHRDPAPRGPARFLPLPGLPPALPEPPGILAPQPPDVGSSDPLSMVTGLEAVRSPSYAS

SEQ ID NO: 36 - protein, 420 aa, Artificial Sequence
  modified FGF21 variant connected to hybrid Fc
ETKTPECPSHTQPLGVFLFPPKPKDTLMISRTPEVTCVVVDVSQEDPEVQFNWYVDGVEVHNAKTKPREEQFNSTYRVVSVLTVLHQDWLNGKEYKCKVSNKGLPSSIEKTISKAKGQPREPQVYTLPPSQEEMTKNQVSLTCLVKGFYPSDIAVEWESNGQPENNYKTTPPVLDSDGSFFLYSRLTVDKSRWQEGNVFSCSVMHEALHNHYTQKSLSLSLGKGGGGSGGGGSGGGGSHPIPDSSPLLQFGGQVRQRYLYTDDAQQTEAHLEIREDGTVGGAADQSPESLLQLKALKPGVIQILGVKTSRFLCQRPDGALYGSLHFDPEACSFREEIRPDGYNVYQSEAHGLPLHLPGNKSPHRDPAPRGPARFLPLPGLPPALPEPPGILAPQPPDVGSSDPLSMVTGLEAVRSPSYES

SEQ ID NO: 37 - protein, 420 aa, Artificial Sequence
  modified FGF21 variant connected to hybrid Fc
ETKTPECPSHTQPLGVFLFPPKPKDTLMISRTPEVTCVVVDVSQEDPEVQFNWYVDGVEVHNAKTKPREEQFNSTYRVVSVLTVLHQDWLNGKEYKCKVSNKGLPSSIEKTISKAKGQPREPQVYTLPPSQEEMTKNQVSLTCLVKGFYPSDIAVEWESNGQPENNYKTTPPVLDSDGSFFLYSRLTVDKSRWQEGNVFSCSVMHEALHNHYTQKSLSLSLGKGGGGSGGGGSGGGGSHPIPDSSPLLQFGGQVRQRYLYTDDAQQTEAHLEIREDGTVGGAADQSPESLLQLKALKPGVIQILGVKTSRFLCQRPDGALYGSLHFDPEACSFREEIRPDGYNVYQSEAHGLPLHLPGNKSPHRDPAPRGPARFLPLPGLPPALPEPPGILAPQPPDVGSSDPLSMVTGLEANRSPSYES

SEQ ID NO: 38 - protein, 419 aa, Artificial Sequence
  modified FGF21 variant connected to hybrid Fc
ETKTPECPSHTQPLGVFLFPPKPKDTLMISRTPEVTCVVVDVSQEDPEVQFNWYVDGVEVHNAKTKPREEQFNSTYRVVSVLTVLHQDWLNGKEYKCKVSNKGLPSSIEKTISKAKGQPREPQVYTLPPSQEEMTKNQVSLTCLVKGFYPSDIAVEWESNGQPENNYKTTPPVLDSDGSFFLYSRLTVDKSRWQEGNVFSCSVMHEALHNHYTQKSLSLSLGKGGGGSGGGGSGGGGSHPIPDSSPLLQFGGQVRQRYLYTDDAQQTEAHLEIREDGTVGGAADQSPESLLQLKALKPGVIQILGVKTSRFLCQRPDGALYGSLHFDPEACSFREEIRPDGYNVYQSEAHGLPLHLPGNKSPHRDPAPRGPARFLPLPGLPPALPEPPGILAPQPPDVGSSDPLSMVNPSQGRSPSYAS

SEQ ID NO: 39 - protein, 419 aa, Artificial Sequence
  modified FGF21 variant connected to hybrid Fc
ETKTPECPSHTQPLGVFLFPPKPKDTLMISRTPEVTCVVVDVSQEDPEVQFNWYVDGVEVHNAKTKPREEQFNSTYRVVSVLTVLHQDWLNGKEYKCKVSNKGLPSSIEKTISKAKGQPREPQVYTLPPSQEEMTKNQVSLTCLVKGFYPSDIAVEWESNGQPENNYKTTPPVLDSDGSFFLYSRLTVDKSRWQEGNVFSCSVMHEALHNHYTQKSLSLSLGKGGGGSGGGGSGGGGSHPIPDSSPLLQFGGQVRQRYLYTDDAQQTEAHLEIREDGTVGGAADQSPESLLQLKALKPGVIQILGVKTSRFLCQRPDGALYGSLHFDPEACSFREEIRPDGYNVYQSEAHGLPLHLPGNKSPHRDPAPRGPARFLPLPGLPPALPEPPGILAPQPPDVGSSDPLSMVNPSQGRSPSYES

SEQ ID NO: 40 - protein, 423 aa, Artificial Sequence
  REG(Amgen)
DKTHTCPPCPAPELLGGPSVFLFPPKPKDTLMISRTPEVTCVVVDVSHEDPEVKFNWYVDGVEVHNAKTKPREEQYNSTYRVVSVLTVLHQDWLNGKEYKCKVSNKALPAPIEKTISKAKGQPREPQVYTLPPSRDELTKNQVSLTCLVKGFYPSDIAVEWESNGQPENNYKTTPPVLDSDGSFFLYSKLTVDKSRWQQGNVFSCSVMHEALHNHYTQKSLSLSPGKGGGGSGGGGSGGGGSHPIPDSSPLLQFGGQVRQRYLYTDDAQQTEAHLEIREDGTVGGAADQSPESLLQLKALKPGVIQILGVKTSRFLCQRPDGALYGSLHFDPEACSFRERLLEDGYNVYQSEAHGLPLHLPGNKSPHRDPAPRGPARFLPLPGLPPALPEPPGILAPQPPDVGSSDPLSMVGGSQGRSPSYES

SEQ ID NO: 41 - protein, 424 aa, Artificial Sequence
  FGF21 connected to Fc(lilly)
ESKYGPPCPPCPAPEAAGGPSVFLFPPKPKDTLMISRTPEVTCVVVDVSQEDPEVQFNWYVDGVEVHNAKTKPREEQFNSTYRVVSVLTVLHQDWLNGKEYKCKVSNKGLPSSIEKTISKAKGQPREPQVYTLPPSQEEMTKNQVSLTCLVKGFYPSDIAVEWESNGQPENNYKTTPPVLDSDGSFFLYSRLTVDKSRWQEGNVFSCSVMHEALHNHYTQKSLSLSLGGGGGSGGGGSGGGGSAHPIPDSSPLLQFGGQVRQRYLYTDDAQQTECHLEIREDGTVGCAADQSPESLLQLKALKPGVIQILGVKTSRFLCQRPDGALYGSLHFDPEACSFREDLKEDGYNVYQSEAHGLPLHLPGDKSPHRKPAPRGPARFLPLPGLPPALPEPPGILAPQPPDVGSSDPLRLVEPSQLRSPSFE

SEQ ID NO: 42 - protein, 31 aa, Artificial Sequence
  GLP-1
HAEGTFTSDVSSYLEGQAAKEFIAWLVKGRG

SEQ ID NO: 43 - protein, 31 aa, Artificial Sequence
  GLP-1 variant
HGEGTFTSDVSSYLEGQAAKEFIAWLVKGRG

SEQ ID NO: 44 - protein, 31 aa, Artificial Sequence
  GLP-1 variant
HGEGTFTSDVSSYLEEQAAKEFIAWLVKGRG

SEQ ID NO: 45 - protein, 31 aa, Artificial Sequence
  GLP-1 variant
HGEGTFTSDVSSYLEGQAAKEFIAWLVKGGG

SEQ ID NO: 46 - protein, 31 aa, Artificial Sequence
  GLP-1 variant
HGEGTFTSDVSSYLEEQAAKEFIAWLVKGGG

SEQ ID NO: 47 - protein, 245 aa, Artificial Sequence
  hybrid Fc5
RNTGRGGEEKKKEKEKEEQEERETKTPECPSHTQPLGVFLFPPKPKDTLMISRTPEVTCVVVDVSQEDPEVQFNWYVDGVEVHNAKTKPREEQFNSTYRVVSVLTVLHQDWLNGKEYKCKVSNKGLPSSIEKTISKAKGQPREPQVYTLPPSQEEMTKNQVSLTCLVKGFYPSDIAVEWESNGQPENNYKTTPPVLDSDGSFFLYSRLTVDKSRWQEGNVFSCSVMHEALHNHYTQKSLSLSLGK

SEQ ID NO: 48 - protein, 233 aa, Artificial Sequence
  hybrid Fc40
EKEKEEQEERETKTPECPSHTQPLGVFLFPPKPKDTLMISRTPEVTCVVVDVSQEDPEVQFNWYVDGVEVHNAKTKPREEQFNSTYRVVSVLTVLHQDWLNGKEYKCKVSNKGLPSSIEKTISKAKGQPREPQVYTLPPSQEEMTKNQVSLTCLVKGFYPSDIAVEWESNGQPENNYKTTPPVLDSDGSFFLYSRLTVDKSRWQEGNVFSCSVMHEALHNHYTQKSLSLSLGK

SEQ ID NO: 49 - protein, 276 aa, Artificial Sequence
  GLP-1 variant connected to hybrid Fc5
HGEGTFTSDVSSYLEGQAAKEFIAWLVKGRGRNTGRGGEEKKKEKEKEEQEERETKTPECPSHTQPLGVFLFPPKPKDTLMISRTPEVTCVVVDVSQEDPEVQFNWYVDGVEVHNAKTKPREEQFNSTYRVVSVLTVLHQDWLNGKEYKCKVSNKGLPSSIEKTISKAKGQPREPQVYTLPPSQEEMTKNQVSLTCLVKGFYPSDIAVEWESNGQPENNYKTTPPVLDSDGSFFLYSRLTVDKSRWQEGNVFSCSVMHEALHNHYTQKSLSLSLGK

SEQ ID NO: 50 - protein, 264 aa, Artificial Sequence
  GLP-1 variant connected to hybrid Fc40
HGEGTFTSDVSSYLEGQAAKEFIAWLVKGRGEKEKEEQEERETKTPECPSHTQPLGVFLFPPKPKDTLMISRTPEVTCVVVDVSQEDPEVQFNWYVDGVEVHNAKTKPREEQFNSTYRVVSVLTVLHQDWLNGKEYKCKVSNKGLPSSIEKTISKAKGQPREPQVYTLPPSQEEMTKNQVSLTCLVKGFYPSDIAVEWESNGQPENNYKTTPPVLDSDGSFFLYSRLTVDKSRWQEGNVFSCSVMHEALHNHYTQKSLSLSLGK

SEQ ID NO: 51 - protein, 276 aa, Artificial Sequence
  GLP-1 variant connected to hybrid Fc5
HGEGTFTSDVSSYLEEQAAKEFIAWLVKGRGRNTGRGGEEKKKEKEKEEQEERETKTPECPSHTQPLGVFLFPPKPKDTLMISRTPEVTCVVVDVSQEDPEVQFNWYVDGVEVHNAKTKPREEQFNSTYRVVSVLTVLHQDWLNGKEYKCKVSNKGLPSSIEKTISKAKGQPREPQVYTLPPSQEEMTKNQVSLTCLVKGFYPSDIAVEWESNGQPENNYKTTPPVLDSDGSFFLYSRLTVDKSRWQEGNVFSCSVMHEALHNHYTQKSLSLSLGK

SEQ ID NO: 52 - protein, 264 aa, Artificial Sequence
  GLP-1 variant connected to hybrid Fc40
HGEGTFTSDVSSYLEEQAAKEFIAWLVKGRGEKEKEEQEERETKTPECPSHTQPLGVFLFPPKPKDTLMISRTPEVTCVVVDVSQEDPEVQFNWYVDGVEVHNAKTKPREEQFNSTYRVVSVLTVLHQDWLNGKEYKCKVSNKGLPSSIEKTISKAKGQPREPQVYTLPPSQEEMTKNQVSLTCLVKGFYPSDIAVEWESNGQPENNYKTTPPVLDSDGSFFLYSRLTVDKSRWQEGNVFSCSVMHEALHNHYTQKSLSLSLGK

SEQ ID NO: 53 - protein, 276 aa, Artificial Sequence
  GLP-1 variant connected to hybrid Fc5
HGEGTFTSDVSSYLEGQAAKEFIAWLVKGGGRNTGRGGEEKKKEKEKEEQEERETKTPECPSHTQPLGVFLFPPKPKDTLMISRTPEVTCVVVDVSQEDPEVQFNWYVDGVEVHNAKTKPREEQFNSTYRVVSVLTVLHQDWLNGKEYKCKVSNKGLPSSIEKTISKAKGQPREPQVYTLPPSQEEMTKNQVSLTCLVKGFYPSDIAVEWESNGQPENNYKTTPPVLDSDGSFFLYSRLTVDKSRWQEGNVFSCSVMHEALHNHYTQKSLSLSLGK

SEQ ID NO: 54 - protein, 264 aa, Artificial Sequence
  GLP-1 variant connected to hybrid Fc40
HGEGTFTSDVSSYLEGQAAKEFIAWLVKGGGEKEKEEQEERETKTPECPSHTQPLGVFLFPPKPKDTLMISRTPEVTCVVVDVSQEDPEVQFNWYVDGVEVHNAKTKPREEQFNSTYRVVSVLTVLHQDWLNGKEYKCKVSNKGLPSSIEKTISKAKGQPREPQVYTLPPSQEEMTKNQVSLTCLVKGFYPSDIAVEWESNGQPENNYKTTPPVLDSDGSFFLYSRLTVDKSRWQEGNVFSCSVMHEALHNHYTQKSLSLSLGK

SEQ ID NO: 55 - protein, 276 aa, Artificial Sequence
  GLP-1 variant connected to hybrid Fc5
HGEGTFTSDVSSYLEEQAAKEFIAWLVKGGGRNTGRGGEEKKKEKEKEEQEERETKTPECPSHTQPLGVFLFPPKPKDTLMISRTPEVTCVVVDVSQEDPEVQFNWYVDGVEVHNAKTKPREEQFNSTYRVVSVLTVLHQDWLNGKEYKCKVSNKGLPSSIEKTISKAKGQPREPQVYTLPPSQEEMTKNQVSLTCLVKGFYPSDIAVEWESNGQPENNYKTTPPVLDSDGSFFLYSRLTVDKSRWQEGNVFSCSVMHEALHNHYTQKSLSLSLGK

SEQ ID NO: 56 - protein, 264 aa, Artificial Sequence
  GLP-1 variant connected to hybrid Fc40
HGEGTFTSDVSSYLEEQAAKEFIAWLVKGGGEKEKEEQEERETKTPECPSHTQPLGVFLFPPKPKDTLMISRTPEVTCVVVDVSQEDPEVQFNWYVDGVEVHNAKTKPREEQFNSTYRVVSVLTVLHQDWLNGKEYKCKVSNKGLPSSIEKTISKAKGQPREPQVYTLPPSQEEMTKNQVSLTCLVKGFYPSDIAVEWESNGQPENNYKTTPPVLDSDGSFFLYSRLTVDKSRWQEGNVFSCSVMHEALHNHYTQKSLSLSLGK

SEQ ID NO: 57 - protein, 275 aa, Artificial Sequence
  Dulaglutide
HGEGTFTSDVSSYLEEQAAKEFIAWLVKGGGGGGGSGGGGSGGGGSAESKYGPPCPPCPAPEAAGGPSVFLFPPKPKDTLMISRTPEVTCVVVDVSQEDPEVQFNWYVDGVEVHNAKTKPREEQFNSTYRVVSVLTVLHQDWLNGKEYKCKVSNKGLPSSIEKTISKAKGQPREPQVYTLPPSQEEMTKNQVSLTCLVKGFYPSDIAVEWESNGQPENNYKTTPPVLDSDGSFFLYSRLTVDKSRWQEGNVFSCSVMHEALHNHYTQKSLSLSLG

SEQ ID NO: 58 - protein, 461 aa, Artificial Sequence
  GLP1(A2G)-HyFc40-GS3-FGF21(EIRP, TGLEAV)
HGEGTFTSDVSSYLEGQAAKEFIAWLVKGRGEKEKEEQEERETKTPECPSHTQPLGVFLFPPKPKDTLMISRTPEVTCVVVDVSQEDPEVQFNWYVDGVEVHNAKTKPREEQFNSTYRVVSVLTVLHQDWLNGKEYKCKVSNKGLPSSIEKTISKAKGQPREPQVYTLPPSQEEMTKNQVSLTCLVKGFYPSDIAVEWESNGQPENNYKTTPPVLDSDGSFFLYSRLTVDKSRWQEGNVFSCSVMHEALHNHYTQKSLSLSLGKGGGGSGGGGSGGGGSHPIPDSSPLLQFGGQVRQRYLYTDDAQQTEAHLEIREDGTVGGAADQSPESLLQLKALKPGVIQILGVKTSRFLCQRPDGALYGSLHFDPEACSFREEIRPDGYNVYQSEAHGLPLHLPGNKSPHRDPAPRGPARFLPLPGLPPALPEPPGILAPQPPDVGSSDPLSMVTGLEAVRSPSYAS

SEQ ID NO: 59 - protein, 473 aa, Artificial Sequence
  GLP1(GE)-HyFc5-GS3-FGF21(EIRP, TGLEAV)
HGEGTFTSDVSSYLEEQAAKEFIAWLVKGRGRNTGRGGEEKKKEKEKEEQEERETKTPECPSHTQPLGVFLFPPKPKDTLMISRTPEVTCVVVDVSQEDPEVQFNWYVDGVEVHNAKTKPREEQFNSTYRVVSVLTVLHQDWLNGKEYKCKVSNKGLPSSIEKTISKAKGQPREPQVYTLPPSQEEMTKNQVSLTCLVKGFYPSDIAVEWESNGQPENNYKTTPPVLDSDGSFFLYSRLTVDKSRWQEGNVFSCSVMHEALHNHYTQKSLSLSLGKGGGGSGGGGSGGGGSHPIPDSSPLLQFGGQVRQRYLYTDDAQQTEAHLEIREDGTVGGAADQSPESLLQLKALKPGVIQILGVKTSRFLCQRPDGALYGSLHFDPEACSFREEIRPDGYNVYQSEAHGLPLHLPGNKSPHRDPAPRGPARFLPLPGLPPALPEPPGILAPQPPDVGSSDPLSMVTGLEAVRSPSYAS

SEQ ID NO: 60 - protein, 461 aa, Artificial Sequence
  GLP1(GE)-HyFc40-GS3-FGF21(EIRP, TGLEAV)
HGEGTFTSDVSSYLEEQAAKEFIAWLVKGRGEKEKEEQEERETKTPECPSHTQPLGVFLFPPKPKDTLMISRTPEVTCVVVDVSQEDPEVQFNWYVDGVEVHNAKTKPREEQFNSTYRVVSVLTVLHQDWLNGKEYKCKVSNKGLPSSIEKTISKAKGQPREPQVYTLPPSQEEMTKNQVSLTCLVKGFYPSDIAVEWESNGQPENNYKTTPPVLDSDGSFFLYSRLTVDKSRWQEGNVFSCSVMHEALHNHYTQKSLSLSLGKGGGGSGGGGSGGGGSHPIPDSSPLLQFGGQVRQRYLYTDDAQQTEAHLEIREDGTVGGAADQSPESLLQLKALKPGVIQILGVKTSRFLCQRPDGALYGSLHFDPEACSFREEIRPDGYNVYQSEAHGLPLHLPGNKSPHRDPAPRGPARFLPLPGLPPALPEPPGILAPQPPDVGSSDPLSMVTGLEAVRSPSYAS

SEQ ID NO: 61 - protein, 473 aa, Artificial Sequence
  GLP1(GG)-HyFc5-GS3-FGF21(EIRP, TGLEAV)
HGEGTFTSDVSSYLEGQAAKEFIAWLVKGGGRNTGRGGEEKKKEKEKEEQEERETKTPECPSHTQPLGVFLFPPKPKDTLMISRTPEVTCVVVDVSQEDPEVQFNWYVDGVEVHNAKTKPREEQFNSTYRVVSVLTVLHQDWLNGKEYKCKVSNKGLPSSIEKTISKAKGQPREPQVYTLPPSQEEMTKNQVSLTCLVKGFYPSDIAVEWESNGQPENNYKTTPPVLDSDGSFFLYSRLTVDKSRWQEGNVFSCSVMHEALHNHYTQKSLSLSLGKGGGGSGGGGSGGGGSHPIPDSSPLLQFGGQVRQRYLYTDDAQQTEAHLEIREDGTVGGAADQSPESLLQLKALKPGVIQILGVKTSRFLCQRPDGALYGSLHFDPEACSFREEIRPDGYNVYQSEAHGLPLHLPGNKSPHRDPAPRGPARFLPLPGLPPALPEPPGILAPQPPDVGSSDPLSMVTGLEAVRSPSYAS

SEQ ID NO: 62 - protein, 461 aa, Artificial Sequence
  GLP1(GG)-HyFc40-GS3-FGF21(EIRP, TGLEAV)
HGEGTFTSDVSSYLEGQAAKEFIAWLVKGGGEKEKEEQEERETKTPECPSHTQPLGVFLFPPKPKDTLMISRTPEVTCVVVDVSQEDPEVQFNWYVDGVEVHNAKTKPREEQFNSTYRVVSVLTVLHQDWLNGKEYKCKVSNKGLPSSIEKTISKAKGQPREPQVYTLPPSQEEMTKNQVSLTCLVKGFYPSDIAVEWESNGQPENNYKTTPPVLDSDGSFFLYSRLTVDKSRWQEGNVFSCSVMHEALHNHYTQKSLSLSLGKGGGGSGGGGSGGGGSHPIPDSSPLLQFGGQVRQRYLYTDDAQQTEAHLEIREDGTVGGAADQSPESLLQLKALKPGVIQILGVKTSRFLCQRPDGALYGSLHFDPEACSFREEIRPDGYNVYQSEAHGLPLHLPGNKSPHRDPAPRGPARFLPLPGLPPALPEPPGILAPQPPDVGSSDPLSMVTGLEAVRSPSYAS

SEQ ID NO: 63 - protein, 473 aa, Artificial Sequence
  GLP1(GEG)-HyFc5-GS3-FGF21(EIRP, TGLEAV)
HGEGTFTSDVSSYLEEQAAKEFIAWLVKGGGRNTGRGGEEKKKEKEKEEQEERETKTPECPSHTQPLGVFLFPPKPKDTLMISRTPEVTCVVVDVSQEDPEVQFNWYVDGVEVHNAKTKPREEQFNSTYRVVSVLTVLHQDWLNGKEYKCKVSNKGLPSSIEKTISKAKGQPREPQVYTLPPSQEEMTKNQVSLTCLVKGFYPSDIAVEWESNGQPENNYKTTPPVLDSDGSFFLYSRLTVDKSRWQEGNVFSCSVMHEALHNHYTQKSLSLSLGKGGGGSGGGGSGGGGSHPIPDSSPLLQFGGQVRQRYLYTDDAQQTEAHLEIREDGTVGGAADQSPESLLQLKALKPGVIQILGVKTSRFLCQRPDGALYGSLHFDPEACSFREEIRPDGYNVYQSEAHGLPLHLPGNKSPHRDPAPRGPARFLPLPGLPPALPEPPGILAPQPPDVGSSDPLSMVTGLEAVRSPSYAS

SEQ ID NO: 64 - protein, 461 aa, Artificial Sequence
  GLP1(GEG)-HyFc40-GS3-FGF21(EIRP, TGLEAV)
HGEGTFTSDVSSYLEEQAAKEFIAWLVKGGGEKEKEEQEERETKTPECPSHTQPLGVFLFPPKPKDTLMISRTPEVTCVVVDVSQEDPEVQFNWYVDGVEVHNAKTKPREEQFNSTYRVVSVLTVLHQDWLNGKEYKCKVSNKGLPSSIEKTISKAKGQPREPQVYTLPPSQEEMTKNQVSLTCLVKGFYPSDIAVEWESNGQPENNYKTTPPVLDSDGSFFLYSRLTVDKSRWQEGNVFSCSVMHEALHNHYTQKSLSLSLGKGGGGSGGGGSGGGGSHPIPDSSPLLQFGGQVRQRYLYTDDAQQTEAHLEIREDGTVGGAADQSPESLLQLKALKPGVIQILGVKTSRFLCQRPDGALYGSLHFDPEACSFREEIRPDGYNVYQSEAHGLPLHLPGNKSPHRDPAPRGPARFLPLPGLPPALPEPPGILAPQPPDVGSSDPLSMVTGLEAVRSPSYAS

SEQ ID NO: 65 - protein, 461 aa, Artificial Sequence
  GLP1(GEG)-HyFc40-GS3-FGF21(EIRP, TGLEAV, A180E)
HGEGTFTSDVSSYLEEQAAKEFIAWLVKGGGEKEKEEQEERETKTPECPSHTQPLGVFLFPPKPKDTLMISRTPEVTCVVVDVSQEDPEVQFNWYVDGVEVHNAKTKPREEQFNSTYRVVSVLTVLHQDWLNGKEYKCKVSNKGLPSSIEKTISKAKGQPREPQVYTLPPSQEEMTKNQVSLTCLVKGFYPSDIAVEWESNGQPENNYKTTPPVLDSDGSFFLYSRLTVDKSRWQEGNVFSCSVMHEALHNHYTQKSLSLSLGKGGGGSGGGGSGGGGSHPIPDSSPLLQFGGQVRQRYLYTDDAQQTEAHLEIREDGTVGGAADQSPESLLQLKALKPGVIQILGVKTSRFLCQRPDGALYGSLHFDPEACSFREEIRPDGYNVYQSEAHGLPLHLPGNKSPHRDPAPRGPARFLPLPGLPPALPEPPGILAPQPPDVGSSDPLSMVTGLEAVRSPSYES

SEQ ID NO: 66 - protein, 461 aa, Artificial Sequence
  GLP1(GEG)-HyFc40-GS3-FGF21(EIRP, TGLEAN, A180E)
HGEGTFTSDVSSYLEEQAAKEFIAWLVKGGGEKEKEEQEERETKTPECPSHTQPLGVFLFPPKPKDTLMISRTPEVTCVVVDVSQEDPEVQFNWYVDGVEVHNAKTKPREEQFNSTYRVVSVLTVLHQDWLNGKEYKCKVSNKGLPSSIEKTISKAKGQPREPQVYTLPPSQEEMTKNQVSLTCLVKGFYPSDIAVEWESNGQPENNYKTTPPVLDSDGSFFLYSRLTVDKSRWQEGNVFSCSVMHEALHNHYTQKSLSLSLGKGGGGSGGGGSGGGGSHPIPDSSPLLQFGGQVRQRYLYTDDAQQTEAHLEIREDGTVGGAADQSPESLLQLKALKPGVIQILGVKTSRFLCQRPDGALYGSLHFDPEACSFREEIRPDGYNVYQSEAHGLPLHLPGNKSPHRDPAPRGPARFLPLPGLPPALPEPPGILAPQPPDVGSSDPLSMVTGLEANRSPSYES

SEQ ID NO: 67 - protein, 460 aa, Artificial Sequence
  GLP1(GEG)-HyFc40-GS3-FGF21(EIRP, G170N, A180E)
HGEGTFTSDVSSYLEEQAAKEFIAWLVKGGGEKEKEEQEERETKTPECPSHTQPLGVFLFPPKPKDTLMISRTPEVTCVVVDVSQEDPEVQFNWYVDGVEVHNAKTKPREEQFNSTYRVVSVLTVLHQDWLNGKEYKCKVSNKGLPSSIEKTISKAKGQPREPQVYTLPPSQEEMTKNQVSLTCLVKGFYPSDIAVEWESNGQPENNYKTTPPVLDSDGSFFLYSRLTVDKSRWQEGNVFSCSVMHEALHNHYTQKSLSLSLGKGGGGSGGGGSGGGGSHPIPDSSPLLQFGGQVRQRYLYTDDAQQTEAHLEIREDGTVGGAADQSPESLLQLKALKPGVIQILGVKTSRFLCQRPDGALYGSLHFDPEACSFREEIRPDGYNVYQSEAHGLPLHLPGNKSPHRDPAPRGPARFLPLPGLPPALPEPPGILAPQPPDVGSSDPLSMVNPSQGRSPSYES

SEQ ID NO: 68 - protein, 4 aa, Artificial Sequence
  FGF21 variant
EIRP

SEQ ID NO: 69 - protein, 6 aa, Artificial Sequence
  FGF21 variant
TGLEAV

SEQ ID NO: 70 - protein, 6 aa, Artificial Sequence
  FGF21 variant
TGLEAN

SEQ ID NO: 71 - DNA, 1383 bp, Artificial Sequence
  nucleic acid molecule coding for DFD23
cacggcgaggggaccttcacaagcgacgtgtcctcttatctggaaggacaggccgctaaggagtttatcgcatggctcgtcaaaggcagaggcgaaaaggagaaggaagagcaggaggagagagaaaccaaaacacccgagtgtcccagtcacactcagcctctgggagtgtttctcttcccacctaagcccaaggatacccttatgatttctaggacacctgaggtgacctgcgtcgttgtggacgtgagtcaagaggacccagaggtccagtttaactggtatgttgacggcgtggaagtgcataatgcaaaaactaaaccccgcgaggaacaattcaattcaacctaccgggtcgtttctgtgttgacagtgctgcatcaagattggctgaacgggaaggagtataagtgtaaagtcagtaataagggactcccctctagtatcgaaaaaactatttcaaaggccaaaggccagcctagagagccacaggtgtacacccttcctccatcccaagaggagatgacaaagaaccaggtgtctctgacttgtctcgtgaaggggttctaccctagtgacatcgctgtcgaatgggagtcaaacggacagccagagaataattataagacaactcctcccgttctggattctgacggcagcttctttctgtactctaggcttactgtggacaaaagtcgctggcaagaagggaacgtcttttcatgttctgttatgcacgaggccttgcacaatcattatacacagaagtctctgagtctctcactgggcaaaggcgggggaggcagcgggggaggcgggtccggaggcgggggatctcatcccatccctgactccagtcctctcctgcaattcgggggccaagtccggcagcggtacctctacacagatgatgctcagcagacagaagcccacctggagatcagggaggatgggaccgtggggggcgctgctgaccagagccccgaaagtctcctgcagctgaaagccttgaagcctggagttattcaaatcttgggagtcaagactagtaggttcctgtgccagcggccagatggggccctgtatggatctctccattttgaccctgaggcctgcagcttccgggaggagatcagacccgacggatacaatgtttaccagtccgaagcccacggcctccctctgcatctgcccgggaacaagtctcctcaccgggaccctgcccccagaggacctgctcgcttcctgccactcccaggcctgccccccgcattgcctgagccacccggaatcctggccccccagccccctgatgtgggatcctctgaccctctgagcatggtgacaggcctggaggccgtgagaagccccagctacgcttcc

SEQ ID NO: 72 - DNA, 1419 bp, Artificial Sequence
  nucleic acid molecule coding for DFD24
cacggcgaggggaccttcacaagcgacgtgtcctcttacctggaagagcaggccgctaaggaatttatcgcatggctcgtcaaaggaagagggaggaacaccggacggggcggggaagagaagaagaaagaaaaggagaaggaagagcaggaggagagagaaaccaaaacacccgagtgtcccagtcacactcagcctctgggagtgtttctcttcccacctaagcccaaggatacccttatgatttctaggacacctgaggtgacctgcgtcgttgtggacgtgagtcaagaggacccagaggtccagtttaactggtatgttgacggcgtggaagtgcataatgcaaaaactaaaccccgcgaggaacaattcaattcaacctaccgggtcgtttctgtgttgacagtgctgcatcaagattggctgaacgggaaggagtataagtgtaaagtcagtaataagggactcccctctagtatcgaaaaaactatttcaaaggccaaaggccagcctagagagccacaggtgtacacccttcctccatcccaagaggagatgacaaagaaccaggtgtctctgacttgtctcgtgaaggggttctaccctagtgacatcgctgtcgaatgggagtcaaacggacagccagagaataattataagacaactcctcccgttctggattctgacggcagcttctttctgtactctaggcttactgtggacaaaagtcgctggcaagaagggaacgtcttttcatgttctgttatgcacgaggccttgcacaatcattatacacagaagtctctgagtctctcactgggcaaaggcgggggaggcagcgggggaggcgggtccggaggcgggggatctcatcccatccctgactccagtcctctcctgcaattcgggggccaagtccggcagcggtacctctacacagatgatgctcagcagacagaagcccacctggagatcagggaggatgggaccgtggggggcgctgctgaccagagccccgaaagtctcctgcagctgaaagccttgaagcctggagttattcaaatcttgggagtcaagactagtaggttcctgtgccagcggccagatggggccctgtatggatctctccattttgaccctgaggcctgcagcttccgggaggagatcagacccgacggatacaatgtttaccagtccgaagcccacggcctccctctgcatctgcccgggaacaagtctcctcaccgggaccctgcccccagaggacctgctcgcttcctgccactcccaggcctgccccccgcattgcctgagccacccggaatcctggccccccagccccctgatgtgggatcctctgaccctctgagcatggtgacaggcctggaggccgtgagaagccccagctacgcttcc

SEQ ID NO: 73 - DNA, 1383 bp, Artificial Sequence
  nucleic acid molecule coding for DFD25
cacggcgaggggaccttcacaagcgacgtgtcctcttacctggaagagcaggccgctaaggaatttatcgcatggctcgtcaaaggaagaggggaaaaggagaaggaagagcaggaggagagagaaaccaaaacacccgagtgtcccagtcacactcagcctctgggagtgtttctcttcccacctaagcccaaggatacccttatgatttctaggacacctgaggtgacctgcgtcgttgtggacgtgagtcaagaggacccagaggtccagtttaactggtatgttgacggcgtggaagtgcataatgcaaaaactaaaccccgcgaggaacaattcaattcaacctaccgggtcgtttctgtgttgacagtgctgcatcaagattggctgaacgggaaggagtataagtgtaaagtcagtaataagggactcccctctagtatcgaaaaaactatttcaaaggccaaaggccagcctagagagccacaggtgtacacccttcctccatcccaagaggagatgacaaagaaccaggtgtctctgacttgtctcgtgaaggggttctaccctagtgacatcgctgtcgaatgggagtcaaacggacagccagagaataattataagacaactcctcccgttctggattctgacggcagcttctttctgtactctaggcttactgtggacaaaagtcgctggcaagaagggaacgtcttttcatgttctgttatgcacgaggccttgcacaatcattatacacagaagtctctgagtctctcactgggcaaaggcgggggaggcagcgggggaggcgggtccggaggcgggggatctcatcccatccctgactccagtcctctcctgcaattcgggggccaagtccggcagcggtacctctacacagatgatgctcagcagacagaagcccacctggagatcagggaggatgggaccgtggggggcgctgctgaccagagccccgaaagtctcctgcagctgaaagccttgaagcctggagttattcaaatcttgggagtcaagactagtaggttcctgtgccagcggccagatggggccctgtatggatctctccattttgaccctgaggcctgcagcttccgggaggagatcagacccgacggatacaatgtttaccagtccgaagcccacggcctccctctgcatctgcccgggaacaagtctcctcaccgggaccctgcccccagaggacctgctcgcttcctgccactcccaggcctgccccccgcattgcctgagccacccggaatcctggccccccagccccctgatgtgggatcctctgaccctctgagcatggtgacaggcctggaggccgtgagaagccccagctacgcttcc

SEQ ID NO: 74 - DNA, 1419 bp, Artificial Sequence
  nucleic acid molecule coding for DFD26
cacggcgaggggaccttcacaagcgacgtgtcctcttatctggaaggacaggccgctaaggagtttatcgcatggctcgtcaaaggcggcggcaggaacaccggacggggcggggaagagaagaagaaagaaaaggagaaggaagagcaggaggagagagaaaccaaaacacccgagtgtcccagtcacactcagcctctgggagtgtttctcttcccacctaagcccaaggatacccttatgatttctaggacacctgaggtgacctgcgtcgttgtggacgtgagtcaagaggacccagaggtccagtttaactggtatgttgacggcgtggaagtgcataatgcaaaaactaaaccccgcgaggaacaattcaattcaacctaccgggtcgtttctgtgttgacagtgctgcatcaagattggctgaacgggaaggagtataagtgtaaagtcagtaataagggactcccctctagtatcgaaaaaactatttcaaaggccaaaggccagcctagagagccacaggtgtacacccttcctccatcccaagaggagatgacaaagaaccaggtgtctctgacttgtctcgtgaaggggttctaccctagtgacatcgctgtcgaatgggagtcaaacggacagccagagaataattataagacaactcctcccgttctggattctgacggcagcttctttctgtactctaggcttactgtggacaaaagtcgctggcaagaagggaacgtcttttcatgttctgttatgcacgaggccttgcacaatcattatacacagaagtctctgagtctctcactgggcaaaggcgggggaggcagcgggggaggcgggtccggaggcgggggatctcatcccatccctgactccagtcctctcctgcaattcgggggccaagtccggcagcggtacctctacacagatgatgctcagcagacagaagcccacctggagatcagggaggatgggaccgtggggggcgctgctgaccagagccccgaaagtctcctgcagctgaaagccttgaagcctggagttattcaaatcttgggagtcaagactagtaggttcctgtgccagcggccagatggggccctgtatggatctctccattttgaccctgaggcctgcagcttccgggaggagatcagacccgacggatacaatgtttaccagtccgaagcccacggcctccctctgcatctgcccgggaacaagtctcctcaccgggaccctgcccccagaggacctgctcgcttcctgccactcccaggcctgccccccgcattgcctgagccacccggaatcctggccccccagccccctgatgtgggatcctctgaccctctgagcatggtgacaggcctggaggccgtgagaagccccagctacgcttcc

SEQ ID NO: 75 - DNA, 1383 bp, Artificial Sequence
  nucleic acid molecule coding for DFD27
cacggcgaggggaccttcacaagcgacgtgtcctcttatctggaaggacaggccgctaaggagtttatcgcatggctcgtcaaaggcggcggcgaaaaggagaaggaagagcaggaggagagagaaaccaaaacacccgagtgtcccagtcacactcagcctctgggagtgtttctcttcccacctaagcccaaggatacccttatgatttctaggacacctgaggtgacctgcgtcgttgtggacgtgagtcaagaggacccagaggtccagtttaactggtatgttgacggcgtggaagtgcataatgcaaaaactaaaccccgcgaggaacaattcaattcaacctaccgggtcgtttctgtgttgacagtgctgcatcaagattggctgaacgggaaggagtataagtgtaaagtcagtaataagggactcccctctagtatcgaaaaaactatttcaaaggccaaaggccagcctagagagccacaggtgtacacccttcctccatcccaagaggagatgacaaagaaccaggtgtctctgacttgtctcgtgaaggggttctaccctagtgacatcgctgtcgaatgggagtcaaacggacagccagagaataattataagacaactcctcccgttctggattctgacggcagcttctttctgtactctaggcttactgtggacaaaagtcgctggcaagaagggaacgtcttttcatgttctgttatgcacgaggccttgcacaatcattatacacagaagtctctgagtctctcactgggcaaaggcgggggaggcagcgggggaggcgggtccggaggcgggggatctcatcccatccctgactccagtcctctcctgcaattcgggggccaagtccggcagcggtacctctacacagatgatgctcagcagacagaagcccacctggagatcagggaggatgggaccgtggggggcgctgctgaccagagccccgaaagtctcctgcagctgaaagccttgaagcctggagttattcaaatcttgggagtcaagactagtaggttcctgtgccagcggccagatggggccctgtatggatctctccattttgaccctgaggcctgcagcttccgggaggagatcagacccgacggatacaatgtttaccagtccgaagcccacggcctccctctgcatctgcccgggaacaagtctcctcaccgggaccctgcccccagaggacctgctcgcttcctgccactcccaggcctgccccccgcattgcctgagccacccggaatcctggccccccagccccctgatgtgggatcctctgaccctctgagcatggtgacaggcctggaggccgtgagaagccccagctacgcttcc

SEQ ID NO: 76 - DNA, 1419 bp, Artificial Sequence
  nucleic acid molecule coding for DFD28
cacggcgaggggaccttcacaagcgacgtgtcctcttacctggaagagcaggccgctaaggaatttatcgcatggctcgtcaaaggaggcgggaggaacaccggacggggcggggaagagaagaagaaagaaaaggagaaggaagagcaggaggagagagaaaccaaaacacccgagtgtcccagtcacactcagcctctgggagtgtttctcttcccacctaagcccaaggatacccttatgatttctaggacacctgaggtgacctgcgtcgttgtggacgtgagtcaagaggacccagaggtccagtttaactggtatgttgacggcgtggaagtgcataatgcaaaaactaaaccccgcgaggaacaattcaattcaacctaccgggtcgtttctgtgttgacagtgctgcatcaagattggctgaacgggaaggagtataagtgtaaagtcagtaataagggactcccctctagtatcgaaaaaactatttcaaaggccaaaggccagcctagagagccacaggtgtacacccttcctccatcccaagaggagatgacaaagaaccaggtgtctctgacttgtctcgtgaaggggttctaccctagtgacatcgctgtcgaatgggagtcaaacggacagccagagaataattataagacaactcctcccgttctggattctgacggcagcttctttctgtactctaggcttactgtggacaaaagtcgctggcaagaagggaacgtcttttcatgttctgttatgcacgaggccttgcacaatcattatacacagaagtctctgagtctctcactgggcaaaggcgggggaggcagcgggggaggcgggtccggaggcgggggatctcatcccatccctgactccagtcctctcctgcaattcgggggccaagtccggcagcggtacctctacacagatgatgctcagcagacagaagcccacctggagatcagggaggatgggaccgtggggggcgctgctgaccagagccccgaaagtctcctgcagctgaaagccttgaagcctggagttattcaaatcttgggagtcaagactagtaggttcctgtgccagcggccagatggggccctgtatggatctctccattttgaccctgaggcctgcagcttccgggaggagatcagacccgacggatacaatgtttaccagtccgaagcccacggcctccctctgcatctgcccgggaacaagtctcctcaccgggaccctgcccccagaggacctgctcgcttcctgccactcccaggcctgccccccgcattgcctgagccacccggaatcctggccccccagccccctgatgtgggatcctctgaccctctgagcatggtgacaggcctggaggccgtgagaagccccagctacgcttcc

SEQ ID NO: 77 - DNA, 1383 bp, Artificial Sequence
  nucleic acid molecule coding for DFD29
cacggcgaggggaccttcacaagcgacgtgtcctcttacctggaagagcaggccgctaaggaatttatcgcatggctcgtcaaaggaggcggggaaaaggagaaggaagagcaggaggagagagaaaccaaaacacccgagtgtcccagtcacactcagcctctgggagtgtttctcttcccacctaagcccaaggatacccttatgatttctaggacacctgaggtgacctgcgtcgttgtggacgtgagtcaagaggacccagaggtccagtttaactggtatgttgacggcgtggaagtgcataatgcaaaaactaaaccccgcgaggaacaattcaattcaacctaccgggtcgtttctgtgttgacagtgctgcatcaagattggctgaacgggaaggagtataagtgtaaagtcagtaataagggactcccctctagtatcgaaaaaactatttcaaaggccaaaggccagcctagagagccacaggtgtacacccttcctccatcccaagaggagatgacaaagaaccaggtgtctctgacttgtctcgtgaaggggttctaccctagtgacatcgctgtcgaatgggagtcaaacggacagccagagaataattataagacaactcctcccgttctggattctgacggcagcttctttctgtactctaggcttactgtggacaaaagtcgctggcaagaagggaacgtcttttcatgttctgttatgcacgaggccttgcacaatcattatacacagaagtctctgagtctctcactgggcaaaggcgggggaggcagcgggggaggcgggtccggaggcgggggatctcatcccatccctgactccagtcctctcctgcaattcgggggccaagtccggcagcggtacctctacacagatgatgctcagcagacagaagcccacctggagatcagggaggatgggaccgtggggggcgctgctgaccagagccccgaaagtctcctgcagctgaaagccttgaagcctggagttattcaaatcttgggagtcaagactagtaggttcctgtgccagcggccagatggggccctgtatggatctctccattttgaccctgaggcctgcagcttccgggaggagatcagacccgacggatacaatgtttaccagtccgaagcccacggcctccctctgcatctgcccgggaacaagtctcctcaccgggaccctgcccccagaggacctgctcgcttcctgccactcccaggcctgccccccgcattgcctgagccacccggaatcctggccccccagccccctgatgtgggatcctctgaccctctgagcatggtgacaggcctggaggccgtgagaagccccagctacgcttcc

SEQ ID NO: 78 - DNA, 1383 bp, Artificial Sequence
  nucleic acid molecule coding for DFD69
cacggcgaggggaccttcacaagcgacgtgtcctcttacctggaagagcaggccgctaaggaatttatcgcatggctcgtcaaaggaggcggggaaaaggagaaggaagagcaggaggagagagaaaccaaaacacccgagtgtcccagtcacactcagcctctgggagtgtttctcttcccacctaagcccaaggatacccttatgatttctaggacacctgaggtgacctgcgtcgttgtggacgtgagtcaagaggacccagaggtccagtttaactggtatgttgacggcgtggaagtgcataatgcaaaaactaaaccccgcgaggaacaattcaattcaacctaccgggtcgtttctgtgttgacagtgctgcatcaagattggctgaacgggaaggagtataagtgtaaagtcagtaataagggactcccctctagtatcgaaaaaactatttcaaaggccaaaggccagcctagagagccacaggtgtacacccttcctccatcccaagaggagatgacaaagaaccaggtgtctctgacttgtctcgtgaaggggttctaccctagtgacatcgctgtcgaatgggagtcaaacggacagccagagaataattataagacaactcctcccgttctggattctgacggcagcttctttctgtactctaggcttactgtggacaaaagtcgctggcaagaagggaacgtcttttcatgttctgttatgcacgaggccttgcacaatcattatacacagaagtctctgagtctctcactgggcaaaggcgggggaggcagcgggggaggcgggtccggaggcgggggatctcatcccatccctgactccagtcctctcctgcaattcgggggccaagtccggcagcggtacctctacacagatgatgctcagcagacagaagcccacctggagatcagggaggatgggaccgtggggggcgctgctgaccagagccccgaaagtctcctgcagctgaaagccttgaagcctggagttattcaaatcttgggagtcaagactagtaggttcctgtgccagcggccagatggggccctgtatggatctctccattttgaccctgaggcctgcagcttccgggaggagatcagacccgacggatacaatgtttaccagtccgaagcccacggcctccctctgcatctgcccgggaacaagtctcctcaccgggaccctgcccccagaggacctgctcgcttcctgccactcccaggcctgccccccgcattgcctgagccacccggaatcctggccccccagccccctgatgtgggatcctctgaccctctgagcatggtgacaggcctggaggccgtgagaagccccagctacgagtcc

SEQ ID NO: 79 - DNA, 1383 bp, Artificial Sequence
  nucleic acid molecule coding for DFD112
cacggcgaggggaccttcacaagcgacgtgtcctcttacctggaagagcaggccgctaaggaatttatcgcatggctcgtcaaaggaggcggggaaaaggagaaggaagagcaggaggagagagaaaccaaaacacccgagtgtcccagtcacactcagcctctgggagtgtttctcttcccacctaagcccaaggatacccttatgatttctaggacacctgaggtgacctgcgtcgttgtggacgtgagtcaagaggacccagaggtccagtttaactggtatgttgacggcgtggaagtgcataatgcaaaaactaaaccccgcgaggaacaattcaattcaacctaccgggtcgtttctgtgttgacagtgctgcatcaagattggctgaacgggaaggagtataagtgtaaagtcagtaataagggactcccctctagtatcgaaaaaactatttcaaaggccaaaggccagcctagagagccacaggtgtacacccttcctccatcccaagaggagatgacaaagaaccaggtgtctctgacttgtctcgtgaaggggttctaccctagtgacatcgctgtcgaatgggagtcaaacggacagccagagaataattataagacaactcctcccgttctggattctgacggcagcttctttctgtactctaggcttactgtggacaaaagtcgctggcaagaagggaacgtcttttcatgttctgttatgcacgaggccttgcacaatcattatacacagaagtctctgagtctctcactgggcaaaggcgggggaggcagcgggggaggcgggtccggaggcgggggatctcatcccatccctgactccagtcctctcctgcaattcgggggccaagtccggcagcggtacctctacacagatgatgctcagcagacagaagcccacctggagatcagggaggatgggaccgtggggggcgctgctgaccagagccccgaaagtctcctgcagctgaaagccttgaagcctggagttattcaaatcttgggagtcaagactagtaggttcctgtgccagcggccagatggggccctgtatggatctctccattttgaccctgaggcctgcagcttccgggaggagatcagacccgacggatacaatgtttaccagtccgaagcccacggcctccctctgcatctgcccgggaacaagtctcctcaccgggaccctgcccccagaggacctgctcgcttcctgccactcccaggcctgccccccgcattgcctgagccacccggaatcctggccccccagccccctgatgtgggatcctctgaccctctgagcatggtgacaggcctggaggccaacagaagccccagctacgagtcc

SEQ ID NO: 80 - DNA, 1380 bp, Artificial Sequence
  nucleic acid molecule coding for DFD114
cacggcgaggggaccttcacaagcgacgtgtcctcttacctggaagagcaggccgctaaggaatttatcgcatggctcgtcaaaggaggcggggaaaaggagaaggaagagcaggaggagagagaaaccaaaacacccgagtgtcccagtcacactcagcctctgggagtgtttctcttcccacctaagcccaaggatacccttatgatttctaggacacctgaggtgacctgcgtcgttgtggacgtgagtcaagaggacccagaggtccagtttaactggtatgttgacggcgtggaagtgcataatgcaaaaactaaaccccgcgaggaacaattcaattcaacctaccgggtcgtttctgtgttgacagtgctgcatcaagattggctgaacgggaaggagtataagtgtaaagtcagtaataagggactcccctctagtatcgaaaaaactatttcaaaggccaaaggccagcctagagagccacaggtgtacacccttcctccatcccaagaggagatgacaaagaaccaggtgtctctgacttgtctcgtgaaggggttctaccctagtgacatcgctgtcgaatgggagtcaaacggacagccagagaataattataagacaactcctcccgttctggattctgacggcagcttctttctgtactctaggcttactgtggacaaaagtcgctggcaagaagggaacgtcttttcatgttctgttatgcacgaggccttgcacaatcattatacacagaagtctctgagtctctcactgggcaaaggcgggggaggcagcgggggaggcgggtccggaggcgggggatctcatcccatccctgactccagtcctctcctgcaattcgggggccaagtccggcagcggtacctctacacagatgatgctcagcagacagaagcccacctggagatcagggaggatgggaccgtggggggcgctgctgaccagagccccgaaagtctcctgcagctgaaagccttgaagcctggagttattcaaatcttgggagtcaagactagtaggttcctgtgccagcggccagatggggccctgtatggatctctccattttgaccctgaggcctgcagcttccgggaggagatcagacccgacggatacaatgtttaccagtccgaagcccacggcctccctctgcatctgcccgggaacaagtctcctcaccgggaccctgcccccagaggacctgctcgcttcctgccactcccaggcctgccccccgcattgcctgagccacccggaatcctggccccccagccccctgatgtgggatcctctgaccctctgagcatggtgaacccttcccagggcagaagccccagctacgagtcc